European Patent Specification EP 3 733 212 B1, published May 21, 2025. Title: Pharmaceutical compositions for preventing or treating pulmonary metastasis of cancer including CHI3L1 inhibitor as active ingredient. Applicant: Industry-University Cooperation Foundation Hanyang University. Application PCT/KR2018/016776. The sequence listing filed with the application follows.

SEQUENCE LISTING (68 sequences)

SEQ ID NO: 1 - RNA, 21 nt, Artificial Sequence
  siChi3l1
caggaguuuaaucucuugcaa

SEQ ID NO: 2 - protein, 44 aa, Artificial Sequence
  dNP2-HA2
KIKKVKKKGRKGSKIKKVKKKGRKGLFGAIAGFIENGWEGMIDG

SEQ ID NO: 3 - DNA, 20 bp, Artificial Sequence
  Actb forward primer
tgtccctgtatgcctctggt

SEQ ID NO: 4 - DNA, 19 bp, Artificial Sequence
  Actb reverse primer written from 5' to 3'
ctctccctttagcacgcac

SEQ ID NO: 5 - DNA, 22 bp, Artificial Sequence
  Chi3l1 forward primer
gtacaagctggtctgctacttc

SEQ ID NO: 6 - DNA, 21 bp, Artificial Sequence
  Chi3l1 reverse primer written from 5' to 3'
cgctgttgtacgaatcgtgta

SEQ ID NO: 7 - DNA, 19 bp, Artificial Sequence
  Tbx21 forward primer
agcaaggacggcgaatgtt

SEQ ID NO: 8 - DNA, 21 bp, Artificial Sequence
  Tbx21 reverse primer written from 5' to 3'
cttggcgaatatacaggtggg

SEQ ID NO: 9 - DNA, 23 bp, Artificial Sequence
  Runx3 forward primer
gactccttccccaactatacacc

SEQ ID NO: 10 - DNA, 20 bp, Artificial Sequence
  Runx3 reverse primer written from 5' to 3'
aagtatgctctgggctcgtg

SEQ ID NO: 11 - DNA, 21 bp, Artificial Sequence
  Ifng forward primer
atgaacgctacacactgcatc

SEQ ID NO: 12 - DNA, 21 bp, Artificial Sequence
  Ifng reverse primer written from 5' to 3'
ctccttgaccgttttcctacc

SEQ ID NO: 13 - DNA, 21 bp, Artificial Sequence
  Gata3 forward primer
gaaggcatccagacccgaaac

SEQ ID NO: 14 - DNA, 20 bp, Artificial Sequence
  Gata3 reverse primer written from 5' to 3'
cgtaccagtggcggtaccca

SEQ ID NO: 15 - DNA, 20 bp, Artificial Sequence
  Il4 forward primer
ggtctcaacccccagctagt

SEQ ID NO: 16 - DNA, 23 bp, Artificial Sequence
  Il4 reverse primer written from 5' to 3'
tagtgaactctctctagtagccg

SEQ ID NO: 17 - DNA, 21 bp, Artificial Sequence
  Il13 forward primer
cagcctccccgataccaaaat

SEQ ID NO: 18 - DNA, 22 bp, Artificial Sequence
  Il13 reverse primer written from 5' to 3'
gatgtgtttcgttgacaaagcg

SEQ ID NO: 19 - DNA, 23 bp, Artificial Sequence
  Il5 forward primer
ctctgttgacaagcaatgagacg

SEQ ID NO: 20 - DNA, 22 bp, Artificial Sequence
  Il5 reverse primer written from 5' to 3'
gtccccgatctgtatgacttct

SEQ ID NO: 21 - DNA, 21 bp, Artificial Sequence
  Il10 forward primer
gctcttactgactggcatgag

SEQ ID NO: 22 - DNA, 20 bp, Artificial Sequence
  Il10 reverse primer written from 5' to 3'
gtgtacgaggatctcgacgc

SEQ ID NO: 23 - DNA, 20 bp, Artificial Sequence
  Junb forward primer
tcacgacgactcttacgcag

SEQ ID NO: 24 - DNA, 20 bp, Artificial Sequence
  Junb reverse primer written from 5' to 3'
agggatagccccagagttcc

SEQ ID NO: 25 - DNA, 21 bp, Artificial Sequence
  Rorgt forward primer
gacccacacctcacaaattga

SEQ ID NO: 26 - DNA, 21 bp, Artificial Sequence
  Rorgt reverse primer written from 5' to 3'
tcgtcacattacaccggatga

SEQ ID NO: 27 - DNA, 21 bp, Artificial Sequence
  Il17 forward primer
tttaactcccttggcgcaaaa

SEQ ID NO: 28 - DNA, 20 bp, Artificial Sequence
  Il17 reverse primer written from 5' to 3'
cacagttacgcctccctttc

SEQ ID NO: 29 - DNA, 21 bp, Artificial Sequence
  Il21 forward primer
ggacccttgtctgtctggtag

SEQ ID NO: 30 - DNA, 23 bp, Artificial Sequence
  Il21 reverse primer
ggacttgaagatagtcgaggtgt

SEQ ID NO: 31 - DNA, 21 bp, Artificial Sequence
  Gmcsf forward primer
ggccttggaagcatgtagagg

SEQ ID NO: 32 - DNA, 23 bp, Artificial Sequence
  Gmcsf reverse primer written from 5' to 3'
ttcagcagagattgctcaagagg

SEQ ID NO: 33 - DNA, 19 bp, Artificial Sequence
  Batf forward primer
gttctgtttctccaggtcc

SEQ ID NO: 34 - DNA, 18 bp, Artificial Sequence
  Batf reverse primer written from 5' to 3'
cgtcgctacgctaagaag

SEQ ID NO: 35 - DNA, 20 bp, Artificial Sequence
  Socs1 forward primer
ctgcggcttctattggggac

SEQ ID NO: 36 - DNA, 21 bp, Artificial Sequence
  Socs1 reverse primer written from 5' to 3'
gctctggaagctgacggaaaa

SEQ ID NO: 37 - DNA, 21 bp, Artificial Sequence
  Socs3 forward primer
atggtcacccacagcaagttt

SEQ ID NO: 38 - DNA, 21 bp, Artificial Sequence
  Socs3 reverse primer written from 5' to 3'
tcctctcgcctaagatgacct

SEQ ID NO: 39 - DNA, 21 bp, Artificial Sequence
  Socs5 forward primer
gagggaggaagccgtaatgag

SEQ ID NO: 40 - DNA, 19 bp, Artificial Sequence
  Socs5 reverse primer written from 5' to 3'
gccttggttttgacacggc

SEQ ID NO: 41 - DNA, 20 bp, Artificial Sequence
  Perforin forward primer
gagaagacctatcaggacca

SEQ ID NO: 42 - DNA, 17 bp, Artificial Sequence
  Perforin reverse primer written from 5' to 3'
gtacgaatggtgtccga

SEQ ID NO: 43 - DNA, 18 bp, Artificial Sequence
  Gzmb forward primer
cctcctgctactgctgac

SEQ ID NO: 44 - DNA, 19 bp, Artificial Sequence
  Gzmb reverse primer written from 5' to 3'
ctctcctgaaacacgactg

SEQ ID NO: 45 - DNA, 22 bp, Artificial Sequence
  Il13ra2 forward primer
accgaaatgttgatagcgacag

SEQ ID NO: 46 - DNA, 22 bp, Artificial Sequence
  Il13ra2 reverse primer written from 5' to 3'
atgcgtaaacagtctcgtaaca

SEQ ID NO: 47 - DNA, 20 bp, Artificial Sequence
  Chit1 forward primer
tgggcaggtgtgatgactct

SEQ ID NO: 48 - DNA, 21 bp, Artificial Sequence
  Chit1 reverse primer written from 5' to 3'
gtcaagccaagaaagggtccc

SEQ ID NO: 49 - DNA, 21 bp, Artificial Sequence
  Amcase forward primer
ctgcgtcagtatgggtttgat

SEQ ID NO: 50 - DNA, 21 bp, Artificial Sequence
  Amcase reverse primer written from 5' to 3'
gataactctcgttgtccgggt

SEQ ID NO: 51 - DNA, 21 bp, Artificial Sequence
  Ym-1 forward primer
acctgccccgttcagtgccat

SEQ ID NO: 52 - DNA, 23 bp, Artificial Sequence
  Ym-1 reverse primer written from 5' to 3'
gacacctctttctgtaaggttcc

SEQ ID NO: 53 - DNA, 19 bp, Artificial Sequence
  Foxp3 forward primer
cccatccccaggagtcttg

SEQ ID NO: 54 - DNA, 21 bp, Artificial Sequence
  Foxp3 reverse primer written from 5' to 3'
atgtcacggggatcagtacca

SEQ ID NO: 55 - DNA, 22 bp, Artificial Sequence
  Eomes forward primer
tcatcgctgtgacggcctacca

SEQ ID NO: 56 - DNA, 23 bp, Artificial Sequence
  Eomes reverse primer written from 5' to 3'
tgaggtagagggtgcctaagggg

SEQ ID NO: 57 - DNA, 22 bp, Artificial Sequence
  Tnfsf10 forward primer
atggtgatttgcatagtgctcc

SEQ ID NO: 58 - DNA, 21 bp, Artificial Sequence
  Tnfsf10 reverse primer written from 5' to 3'
agaacttgtctgggacgaacg

SEQ ID NO: 59 - DNA, 21 bp, Artificial Sequence
  Ccr5 forward primer
ttttcaagggtcagttccgac

SEQ ID NO: 60 - DNA, 22 bp, Artificial Sequence
  Ccr5 reverse primer written from 5' to 3'
cacccattgtactaccagaagg

SEQ ID NO: 61 - DNA, 23 bp, Artificial Sequence
  Cxcr3 forward primer
taccttgaggttagtgaacgtca

SEQ ID NO: 62 - DNA, 22 bp, Artificial Sequence
  Cxcr3 reverse primer written from 5' to 3'
ctaataccccttttgctctcgc

SEQ ID NO: 63 - DNA, 21 bp, Artificial Sequence
  Cxcr2 forward primer
atgccctctattctgccagat

SEQ ID NO: 64 - DNA, 23 bp, Artificial Sequence
  Cxcr2 reverse primer written from 5' to 3'
cagtagaatatgttggcctcgtg

SEQ ID NO: 65 - DNA, 21 bp, Artificial Sequence
  Ctse forward primer
gacatcagtcccttcggaaga

SEQ ID NO: 66 - DNA, 23 bp, Artificial Sequence
  Ctse reverse primer written from 5' to 3'
ataagctcacagttacttgggga

SEQ ID NO: 67 - DNA, 21 bp, Artificial Sequence
  Twist1 forward primer
ggacaagctgagcaagattca

SEQ ID NO: 68 - DNA, 19 bp, Artificial Sequence
  Twist1 reverse primer written from 5' to 3'
gagtcgatgcggaagaggc